European Patent Specification EP 3 469 361 B1, published July 31, 2024. Title: Novel method for identifying deltaT-cell (or gammaT-cell) receptor chains or parts thereof that mediate an anti-tumour or an anti-infective response. Applicant: UMC Utrecht Holding B.V. Gadeta B.V. Albert-Ludwig-Universitat-Freiburg. The sequence listing filed with the application follows.

SEQUENCE LISTING (101 sequences)

SEQ ID NO: 1 - DNA, 19 bp, artificial
  primer: Constant region TRB
cagtatctggagtcattga

SEQ ID NO: 2 - DNA, 17 bp, artificial
  primer: Constant region TRD
cttggatgacacgagat

SEQ ID NO: 3 - DNA, 45 bp, Artificial
  Oligonucleotide
  misc_feature (24)..(27): n is a, c, g, t or u
  misc_feature (29)..(32): n is a, c, g, t or u
  misc_feature (34)..(37): n is a, c, g, t or u
  misc_feature (42)..(45): riboguanosine
aagcaguggtaucaacgcagagunnnnunnnnunnnnucttgggg

SEQ ID NO: 4 - DNA, 21 bp, Artificial
  Primer
tgcttctgatggctcaaacac

SEQ ID NO: 5 - DNA, 20 bp, Artificial
  Primer
aacggatggtttggtatgag

SEQ ID NO: 6 - DNA, 33 bp, Artificial
  Primer
cactctatccgacaagcagtggtatcaacgcag

SEQ ID NO: 7 - protein, 19 aa, Artificial
  peptide, Vd1 Fe11
CALGDSYGGGPLYTDKLIF

SEQ ID NO: 8 - protein, 14 aa, Artificial
  Peptide: Vd2, clone 3
CACDLLGYTDKLIF

SEQ ID NO: 9 - protein, 16 aa, Artificial
  Peptide: Vd2, clone 5
CACDALKRTDTDKLIF

SEQ ID NO: 10 - protein, 13 aa, Artificial
  Peptide: CDR3 gamma chain, Fe11
ATWDRPEIYYKKL

SEQ ID NO: 11 - protein, 15 aa, Artificial
  Peptide: CDR3 gamma chain, clone 3
CALWEEELGKKIKVF

SEQ ID NO: 12 - protein, 16 aa, Artificial
  Peptide: CDR3 gamma chain, clone 5
CALWEIQELGKKIKVF

SEQ ID NO: 13 - protein, 288 aa, Artificial
  TRD Cl3
MERISSLIHLSLFWAGVMSAIELVPEHQTVPVSIGVPATLRCSMKGEAIGNYYINWYRKTQGNTMTFIYREKDIYGPGFKDNFQGDIDIAKNLAVLKILAPSERDEGSYYCACDLLGYTDKLIFGKGTRVTVEPRSQPHTKPSVFVMKNGTNVACLVKEFYPKDIRINLVSSKKITEFDPAIVISPSGKYNAVKLGKYEDSNSVTCSVQHDNKTVHSTDFEVKTDSTDHVKPKETENTKQPSKSCHKPKAIVHTEKVNMMSLTVLGLRMLFAKTVAVNFLLTAKLFFL

SEQ ID NO: 14 - protein, 313 aa, Artificial
  TRG Cl3
MVSLLHASTLAVLGALCVYGAGHLEQPQISSTKTLSKTARLECVVSGITISATSVYWYRERPGEVIQFLVSISYDGTVRKESGIPSGKFEVDRIPETSTSTLTIHNVEKQDIATYYCALWEEELGKKIKVFGPGTKLIITDKQLDADVSPKPTIFLPSIAETKLQKAGTYLCLLEKFFPDVIKIHWEEKKSNTILGSQEGNTMKTNDTYMKFSWLTVPEKSLDKEHRCIVRHENNKNGVDQEIIFPPIKTDVITMDPKDNCSKDANDTLLLQLTNTSAYYMYLLLLLKSVVYFAIITCCLLRRTAFCCNGEKS

SEQ ID NO: 15 - protein, 290 aa, Artificial
  TRD Cl5
MERISSLIHLSLFWAGVMSAIELVPEHQTVPVSIGVPATLRCSMKGEAIGNYYINWYRKTQGNTMTFIYREKDIYGPGFKDNFQGDIDIAKNLAVLKILAPSERDEGSYYCACDALKRTDTDKLIFGKGTRVTVEPRSQPHTKPSVFVMKNGTNVACLVKEFYPKDIRINLVSSKKITEFDPAIVISPSGKYNAVKLGKYEDSNSVTCSVQHDNKTVHSTDFEVKTDSTDHVKPKETENTKQPSKSCHKPKAIVHTEKVNMMSLTVLGLRMLFAKTVAVNFLLTAKLFFL

SEQ ID NO: 16 - protein, 314 aa, Artificial
  TRG Cl5
MVSLLHASTLAVLGALCVYGAGHLEQPQISSTKTLSKTARLECVVSGITISATSVYWYRERPGEVIQFLVSISYDGTVRKESGIPSGKFEVDRIPETSTSTLTIHNVEKQDIATYYCALWEIQELGKKIKVFGPGTKLIITDKQLDADVSPKPTIFLPSIAETKLQKAGTYLCLLEKFFPDVIKIHWEEKKSNTILGSQEGNTMKTNDTYMKFSWLTVPEKSLDKEHRCIVRHENNKNGVDQEIIFPPIKTDVITMDPKDNCSKDANDTLLLQLTNTSAYYMYLLLLLKSVVYFAIITCCLLRRTAFCCNGEKS

SEQ ID NO: 17 - protein, 293 aa, Artificial
  TRD Fe11
MVFSSLLCVFVAFSYSGSSVAQKVTQAQSSVSMPVRKAVTLNCLYETSWWSYYIFWYKQLPSKEMIFLIRQGSDEQNAKSGRYSVNFKKAAKSVALTISALQLEDSAKYFCALGDSYGGGPLYTDKLIFGKGTRVTVEPRSQPHTKPSVFVMKNGTNVACLVKEFYPKDIRINLVSSKKITEFDPAIVISPSGKYNAVKLGKYEDSNSVTCSVQHDNKTVHSTDFEVKTDSTDHVKPKETENTKQPSKSCHKPKAIVHTEKVNMMSLTVLGLRMLFAKTVAVNFLLTAKLFFL

SEQ ID NO: 18 - protein, 309 aa, Artificial
  TRG Fe11
MGWALLVLLAFLSPASQKSSNLEGGTKSVTRPTRSSAEITCDLTVINAFYIHWYLHQEGKAPQRLLYYDVSNSKDVLESGLSPGKYYTHTPRRWSWILILRNLIENDSGVYYCATWDRPEIYYKKLFGSGTTLVVTDKQLDADVSPKPTIFLPSIAETKLQKAGTYLCLLEKFFPDVIKIHWEEKKSNTILGSQEGNTMKTNDTYMKFSWLTVPEKSLDKEHRCIVRHENNKNGVDQEIIFPPIKTDVITMDPKDNCSKDANDTLLLQLTNTSAYYMYLLLLLKSVVYFAIITCCLLRRTAFCCNGEKS

SEQ ID NO: 19 - protein, 14 aa, Artificial
  CDR3  VG4  E113
CATWDGPPYYKKLF

SEQ ID NO: 20 - protein, 11 aa, Artificial
  CDR3  VG2  F4
CATWDGQKKLF

SEQ ID NO: 21 - protein, 11 aa, Artificial
  CDR3  VG8  Zi11
CATWDNYKKLF

SEQ ID NO: 22 - protein, 18 aa, Artificial
  CDR3  VD5  D37
CAASSPIRGYTGSDKLIF

SEQ ID NO: 23 - protein, 18 aa, Artificial
  CDR3  VD5  E113
CAASSPIRGYTGSDKLIF

SEQ ID NO: 24 - protein, 17 aa, Artificial
  CDR3 VD1 F4
CALGELRYWGIVDKLIF

SEQ ID NO: 25 - protein, 25 aa, Artificial
  CDR3 VD1 Zi11
CALGELRGQISFLYLLGDTTDKLIF

SEQ ID NO: 26 - DNA, 895 bp, Homo sapiens
atggccatgctcctgggggcatcagtgctgattctgtggcttcagccagactgggtaaacagtcaacagaagaatgatgaccagcaagttaagcaaaattcaccatccctgagcgtccaggaaggaagaatttctattctgaactgtgactatactaacagcatgtttgattatttcctatggtacaaaaaataccctgctgaaggtcctacattcctgatatctataagttccattaaggataaaaatgaagatggaagattcactgtcttcttaaacaaaagtgccaagcacctctctctgcacattgtgccctcccagcctggagactctgcagtgtacttctgtgcagcaagctcccctattaggggatatacagggtccgataaactcatctttggaaaaggaacccgtgtgactgtggaaccaagaagtcagcctcataccaaaccatccgtttttgtcatgaaaaatggaacaaatgtcgcttgtctggtgaaggaattctaccccaaggatataagaataaatctcgtgtcatccaagaagataacagagtttgatcctgctattgtcatctctcccagtgggaagtacaatgctgtcaagcttggtaaatatgaagattcaaattcagtgacatgttcagttcaacacgacaataaaactgtgcactccactgactttgaagtgaagacagattctacagatcacgtaaaaccaaaggaaactgaaaacacaaagcaaccttcaaagagctgccataaacccaaagccatagttcataccgagaaggtgaacatgatgtccctcacagtgcttgggctacgaatgctgtttgcaaagactgttgccgtcaattttctcttgactgccaagttatttttcttgtaag

SEQ ID NO: 27 - protein, 13 aa, Artificial
  CDR3 VG4 C132
CATWDGFYYKKLF

SEQ ID NO: 28 - protein, 18 aa, Artificial
  CDR3 VD5 C132
CAASSPIRGYTGSDKLIF

SEQ ID NO: 29 - protein, 271 aa, Homo sapiens
DQQVKQNSPSLSVQEGRISILNCDYTNSMFDYFLWYKKYPAEGPTFLISISSIKDKNEDGRFTVFLNKSAKHLSLHIVPSQPGDSAVYFCAASSPIRGYTGSDKLIFGKGTRVTVEPRSQPHTKPSVFVMKNGTNVACLVKEFYPKDIRINLVSSKKITEFDPAIVISPSGKYNAVKLGKYEDSNSVTCSVQHDNKTVHSTDFEVKTDSTDHVKPKETENTKQPSKSCHKPKAIVHTEKVNMMSLTVLGLRMLFAKTVAVNFLLTAKLFFL

SEQ ID NO: 30 - protein, 290 aa, Homo sapiens
SSNLEGRTKSVIRQTGSSAEITCDLAEGSTGYIHWYLHQEGKAPQRLLYYDSYTSSVVLESGISPGKYDTYGSTRKNLRMILRNLIENDSGVYYCATWDGPPYYKKLFGSGTTLVVTDKQLDADVSPKPTIFLPSIAETKLQKAGTYLCLLEKFFPDVIKIHWEEKKSNTILGSQEGNTMKTNDTYMKFSWLTVPEKSLDKEHRCIVRHENNKNGVDQEIIFPPIKTDVITMDPKDNCSKDANDTLLLQLTNTSAYYMYLLLLLKSVVYFAIITCCLLRRTAFCCNGEKS

SEQ ID NO: 31 - protein, 271 aa, Homo sapiens
AQKVTQAQSSVSMPVRKAVTLNCLYETSWWSYYIFWYKQLPSKEMIFLIRQGSDEQNAKSGRYSVNFKKAAKSVALTISALQLEDSAKYFCALGELRYWGIVDKLIFGKGTRVTVEPRSQPHTKPSVFVMKNGTNVACLVKEFYPKDIRINLVSSKKITEFDPAIVISPSGKYNAVKLGKYEDSNSVTCSVQHDNKTVHSTDFEVKTDSTDHVKPKETENTKQPSKSCHKPKAIVHTEKVNMMSLTVLGLRMLFAKTVAVNFLLTAKLFFL

SEQ ID NO: 32 - protein, 287 aa, Homo sapiens
SSNLEGRTKSVIRQTGSSAEITCDLAEGSNGYIHWYLHQEGKAPQRLQYYDSYNSKVVLESGVSPGKYYTYASTRNNLRLILRNLIENDSGVYYCATWDGQKKLFGSGTTLVVTDKQLDADVSPKPTIFLPSIAETKLQKAGTYLCLLEKFFPDVIKIHWEEKKSNTILGSQEGNTMKTNDTYMKFSWLTVPEKSLDKEHRCIVRHENNKNGVDQEIIFPPIKTDVITMDPKDNCSKDANDTLLLQLTNTSAYYMYLLLLLKSVVYFAIITCCLLRRTAFCCNGEKS

SEQ ID NO: 33 - protein, 279 aa, Homo sapiens
AQKVTQAQSSVSMPVRKAVTLNCLYETSWWSYYIFWYKQLPSKEMIFLIRQGSDEQNAKSGRYSVNFKKAAKSVALTISALQLEDSAKYFCALGELRGQISFLYLLGDTTDKLIFGKGTRVTVEPRSQPHTKPSVFVMKNGTNVACLVKEFYPKDIRINLVSSKKITEFDPAIVISPSGKYNAVKLGKYEDSNSVTCSVQHDNKTVHSTDFEVKTDSTDHVKPKETENTKQPSKSCHKPKAIVHTEKVNMMSLTVLGLRMLFAKTVAVNFLLTAKLFFL

SEQ ID NO: 34 - protein, 287 aa, Homo sapiens
SSNLEGRTKSVTRPTGSSAVITCDLPVENAVYTHWYLHQEGKAPQRLLYYDSYNSRVVLESGISREKYHTYASTGKSLKFILENLIERDSGVYYCATWDNYKKLFGSGTTLVVTDKQLDADVSPKPTIFLPSIAETKLQKAGTYLCLLEKFFPDVIKIHWQEKKSNTILGSQEGNTMKTNDTYMKFSWLTVPEKSLDKEHRCIVRHENNKNGVDQEIIFPPIKTDVITMDPKDNCSKDANDTLLLQLTNTSAYYMYLLLLLKSVVYFAIITCCLLRRTAFCCNGEKS

SEQ ID NO: 35 - protein, 271 aa, Homo sapiens; identical to SEQ ID NO: 29

SEQ ID NO: 36 - protein, 287 aa, Homo sapiens
SSNLEGRTKSVTRPTGSSAVITCDLPVENAVYTHWYLHQEGKAPQRLLYYDSYNSRVVLESGISREKYHTYASTGKSLKFILENLIERDSGVYYCATWDNYMKLFGSGTTLVVTDKQLDADVSPKPTIFLPSIAETKLQKAGTYLCLLEKFFPDVIKIHWEEKKSNTILGSQEGNTMKTNDTYMKFSWLTVPEKSLDKEHRCIVRHENNKNGVDQEIIFPPIKTDVITMDPKDNCSKDANDTLLLQLTNTSAYYMYLLLLLKSVVYFAIITCCLLRRTAFCCNGEKS

SEQ ID NO: 37 - protein, 271 aa, Homo sapiens; identical to SEQ ID NO: 29

SEQ ID NO: 38 - protein, 289 aa, Homo sapiens
SSNLEGRTKSVIRQTGSSAEITCDLAEGSTGYIHWYLHQEGKAPQRLLYYDSYTSSVVLESGISPGKYDTYGSTRKNLRMILRNLIENDSGVYYCATWDGFYYKKLFGSGTTLVVTDKQLDADVSPKPTIFLPSIAETKLQKAGTYLCLLEKFFPDVIKIHWEEKKSNTILGSQEGNTMKTNDTYMKFSWLTVPEKSLDKEHRCIVRHENNKNGVDQEIIFPPIKTDVITMDPKDNCSKDANDTLLLQLTNTSAYYMYLLLLLKSVVYFAIITCCLLRRTAFCCNGEKS

SEQ ID NO: 39 - protein, 11 aa, Artificial
  CDR3 VG8 D37
CATWDNYMKLF

SEQ ID NO: 40 - protein, 23 aa, Artificial
  CDR3 VD3 F2
CASSYTLKLGDTPGRVRDWKLIF

SEQ ID NO: 41 - DNA, 924 bp, Homo sapiens
atgcagtgggccctagcggtgcttctagctttcctgtctcctgccagtcagaaatcttccaacttggaagggagaacgaagtcagtcatcaggcagactgggtcatctgctgaaatcacttgtgatcttgctgaaggaagtaccggctacatccactggtacctacaccaggaggggaaggccccacagcgtcttctgtactatgactcctacacctccagcgttgtgttggaatcaggaatcagcccagggaagtatgatacttatggaagcacaaggaagaacttgagaatgatactgcgaaatcttattgaaaatgactctggagtctattactgtgccacctgggatgggcctccttattataagaaactctttggcagtggaacaacactggttgtcacagataaacaacttgatgcagatgtttcccccaagcccactatttttcttccttcaattgctgaaacaaagctccagaaggctggaacatacctttgtcttcttgagaaatttttccctgatgttattaagatacattggcaagaaaagaagagcaacacgattctgggatcccaggaggggaacaccatgaagactaacgacacatacatgaaatttagctggttaacggtgccagaaaagtcactggacaaagaacacagatgtatcgtcagacatgagaataataaaaacggagttgatcaagaaattatctttcctccaataaagacagatgtcatcacaatggatcccaaagacaattgttcaaaagatgcaaatgatacactactgctgcagctcacaaacacctctgcatattacatgtacctcctcctgctcctcaagagtgtggtctattttgccatcatcacctgctgtctgcttagaagaacggctttctgctgcaatggagagaaatca

SEQ ID NO: 42 - DNA, 877 bp, Homo sapiens
atgctgttctccagcctgctgtgtgtatttgtggccttcagctactctggatcaagtgtggcccagaaggttactcaagcccagtcatcagtatccatgccagtgaggaaagcagtcaccctgaactgcctgtatgaaacaagttggtggtcatattatattttttggtacaagcaacttcccagcaaagagatgattttccttattcgccagggttctgatgaacagaatgcaaaaagtggtcgctattctgtcaacttcaagaaagcagcgaaatccgtcgccttaaccatttcagccttacagctagaagattcagcaaagtacttttgtgctcttggggaactccggtactgggggatagtcgataaactcatctttggaaaaggaacccgtgtgactgtggaaccaagaagtcagcctcataccaaaccatccgtttttgtcatgaaaaatggaacaaatgtcgcttgtctggtgaaggaattctaccccaaggatataagaataaatctcgtgtcatccaagaagataacagagtttgatcctgctattgtcatctctcccagtgggaagtacaatgctgtcaagcttggtaaatatgaagattcaaattcagtgacatgttcagttcaacacgacaataaaactgtgcactccactgactttgaagtgaagacagattctacagatcacgtaaaaccaaaggaaactgaaaacacaaagcaaccttcaaagagctgccataaacccaaagccatagttcataccgagaaggtgaacatgatgtccctcacagtgcttgggctacgaatgctgtttgcaaagactgttgccgtcaattttctcttgactgccaagttatttttcttgtaag

SEQ ID NO: 43 - DNA, 915 bp, Homo sapiens
atgcagtgggccctagcggtgcttctagctttcctgtctcctgccagtcagaaatcttccaacttggaagggagaacgaagtcagtcatcaggcagactgggtcatctgctgaaatcacttgtgatcttgctgaaggaagtaacggctacatccactggtacctacaccaggaggggaaggccccacagcgtcttcagtactatgactcctacaactccaaggttgtgttggaatcaggagtcagtccagggaagtattatacttacgcaagcacaaggaacaacttgagattgatactgcgaaatctaattgaaaatgactctggggtctattactgtgccacctgggacgggcaaaagaaactctttggcagtggaacaacactggttgtcacagataaacaacttgatgcagatgtttcccccaagcccactatttttcttccttcaattgctgaaacaaagctccagaaggctggaacatacctttgtcttcttgagaaatttttccctgatgttattaagatacattggcaagaaaagaagagcaacacgattctgggatcccaggaggggaacaccatgaagactaacgacacatacatgaaatttagctggttaacggtgccagaaaagtcactggacaaagaacacagatgtatcgtcagacatgagaataataaaaacggagttgatcaagaaattatctttcctccaataaagacagatgtcatcacaatggatcccaaagacaattgttcaaaagatgcaaatgatacactactgctgcagctcacaaacacctctgcatattacatgtacctcctcctgctcctcaagagtgtggtctattttgccatcatcacctgctgtctgcttagaagaacggctttctgctgcaatggagagaaatca

SEQ ID NO: 44 - DNA, 901 bp, Homo sapiens
atgctgttctccagcctgctgtgtgtatttgtggccttcagctactctggatcaagtgtggcccagaaggttactcaagcccagtcatcagtatccatgccagtgaggaaagcagtcaccctgaactgcctgtatgaaacaagttggtggtcatattatattttttggtacaagcaacttcccagcaaagagatgattttccttattcgccagggttctgatgaacagaatgcaaaaagtggtcgctattctgtcaacttcaagaaagcagcgaaatccgtcgccttaaccatttcagccttacagctagaagattcagcaaagtacttttgtgctcttggggaacttaggggacaaatttccttcctttatttactgggggatacaaccgataaactcatctttggaaaaggaacccgtgtgactgtggaaccaagaagtcagcctcataccaaaccatccgtttttgtcatgaaaaatggaacaaatgtcgcttgtctggtgaaggaattctaccccaaggatataagaataaatctcgtgtcatccaagaagataacagagtttgatcctgctattgtcatctctcccagtgggaagtacaatgctgtcaagcttggtaaatatgaagattcaaattcagtgacatgttcagttcaacacgacaataaaactgtgcactccactgactttgaagtgaagacagattctacagatcacgtaaaaccaaaggaaactgaaaacacaaagcaaccttcaaagagctgccataaacccaaagccatagttcataccgagaaggtgaacatgatgtccctcacagtgcttgggctacgaatgctgtttgcaaagactgttgccgtcaattttctcttgactgccaagttatttttcttgtaag

SEQ ID NO: 45 - DNA, 915 bp, Homo sapiens
atgctgttggctctagctctgcttctagctttcctgcctcctgccagtcagaaatcttccaacttggaagggagaacaaagtcagtcaccaggccaactgggtcatcagctgtaatcacttgtgatcttcctgtagaaaatgccgtctacacccactggtacctacaccaggaggggaaggccccacagcgtcttctgtactatgactcctacaactccagggttgtgttggaatcaggaatcagtcgagaaaagtatcatacttatgcaagcacagggaagagccttaaatttatactggaaaatctaattgaacgtgactctggggtctattactgtgccacctgggataattataagaaactctttggcagtggaacaacactggttgtcacagataaacaacttgatgcagatgtttcccccaagcccactatttttcttccttcaattgctgaaacaaagctccagaaggctggaacatacctttgtcttcttgagaaatttttccctgatgttattaagatacattggcaagaaaagaagagcaacacgattctgggatcccaggaggggaacaccatgaagactaacgacacatacatgaaatttagctggttaacggtgccagaaaagtcactggacaaagaacacagatgtatcgtcagacatgagaataataaaaacggagttgatcaagaaattatctttcctccaataaagacagatgtcatcacaatggatcccaaagacaattgttcaaaagatgcaaatgatacactactgctgcagctcacaaacacctctgcatattacatgtacctcctcctgctcctcaagagtgtggtctattttgccatcatcacctgctgtctgcttagaagaacggctttctgctgcaatggagagaaatca

SEQ ID NO: 46 - DNA, 895 bp, Homo sapiens; identical to SEQ ID NO: 26

SEQ ID NO: 47 - DNA, 915 bp, Homo sapiens
atgctgttggctctagctctgcttctagctttcctgcctcctgccagtcagaaatcttccaacttggaagggagaacaaagtcagtcaccaggccaactgggtcatcagctgtaatcacttgtgatcttcctgtagaaaatgccgtctacacccactggtacctacaccaggaggggaaggccccacagcgtcttctgtactatgactcctacaactccagggttgtgttggaatcaggaatcagtcgagaaaagtatcatacttatgcaagcacagggaagagccttaaatttatactggaaaatctaattgaacgtgactctggggtctattactgtgccacctgggataattatatgaaactctttggcagtggaacaacactggttgtcacagataaacaacttgatgcagatgtttcccccaagcccactatttttcttccttcaattgctgaaacaaagctccagaaggctggaacatacctttgtcttcttgagaaatttttccctgatgttattaagatacattggcaagaaaagaagagcaacacgattctgggatcccaggaggggaacaccatgaagactaacgacacatacatgaaatttagctggttaacggtgccagaaaagtcactggacaaagaacacagatgtatcgtcagacatgagaataataaaaacggagttgatcaagaaattatctttcctccaataaagacagatgtcatcacaatggatcccaaagacaattgttcaaaagatgcaaatgatacactactgctgcagctcacaaacacctctgcatattacatgtacctcctcctgctcctcaagagtgtggtctattttgccatcatcacctgctgtctgcttagaagaacggctttctgctgcaatggagagaaatca

SEQ ID NO: 48 - DNA, 895 bp, Homo sapiens; identical to SEQ ID NO: 26

SEQ ID NO: 49 - DNA, 921 bp, Homo sapiens
atgcagtgggccctagcggtgcttctagctttcctgtctcctgccagtcagaaatcttccaacttggaagggagaacgaagtcagtcatcaggcagactgggtcatctgctgaaatcacttgtgatcttgctgaaggaagtaccggctacatccactggtacctacaccaggaggggaaggccccacagcgtcttctgtactatgactcctacacctccagcgttgtgttggaatcaggaatcagcccagggaagtatgatacttatggaagcacaaggaagaacttgagaatgatactgcgaaatcttattgaaaatgactctggagtctattactgtgccacctgggatggattttattataagaaactctttggcagtggaacaacactggttgtcacagataaacaacttgatgcagatgtttcccccaagcccactatttttcttccttcaattgctgaaacaaagctccagaaggctggaacatacctttgtcttcttgagaaatttttccctgatgttattaagatacattggcaagaaaagaagagcaacacgattctgggatcccaggaggggaacaccatgaagactaacgacacatacatgaaatttagctggttaacggtgccagaaaagtcactggacaaagaacacagatgtatcgtcagacatgagaataataaaaacggagttgatcaagaaattatctttcctccaataaagacagatgtcatcacaatggatcccaaagacaattgttcaaaagatgcaaatgatacactactgctgcagctcacaaacacctctgcatattacatgtacctcctcctgctcctcaagagtgtggtctattttgccatcatcacctgctgtctgcttagaagaacggctttctgctgcaatggagagaaatca

SEQ ID NO: 50 - DNA, 883 bp, Homo sapiens
atgctgttctccagcctgctgtgtgtatttgtggccttcagctactctggatcaagtgtggcccagaaggttactcaagcccagtcatcagtatccatgccagtgaggaaagcagtcaccctgaactgcctgtatgaaacaagttggtggtcatattatattttttggtacaagcaacttcccagcaaagagatgattttccttattcgccagggttctgatgaacagaatgcaaaaagtggtcgctattctgtcaacttcaagaaagcagcgaaatccgtcgccttaaccatttcagccttacagctagaagattcagcaaagtacttttgtgctcttggggattcctacggtgggggacccctatacaccgataaactcatctttggaaaaggaacccgtgtgactgtggaaccaagaagtcagcctcataccaaaccatccgtttttgtcatgaaaaatggaacaaatgtcgcttgtctggtgaaggaattctaccccaaggatataagaataaatctcgtgtcatccaagaagataacagagtttgatcctgctattgtcatctctcccagtgggaagtacaatgctgtcaagcttggtaaatatgaagattcaaattcagtgacatgttcagttcaacacgacaataaaactgtgcactccactgactttgaagtgaagacagattctacagatcacgtaaaaccaaaggaaactgaaaacacaaagcaaccttcaaagagctgccataaacccaaagccatagttcataccgagaaggtgaacatgatgtccctcacagtgcttgggctacgaatgctgtttgcaaagactgttgccgtcaattttctcttgactgccaagttatttttcttgtaag

SEQ ID NO: 51 - DNA, 927 bp, Homo sapiens
atgcggtgggccctactggtgcttctagctttcctgtctcctgccagtcagaaatcttccaacttggaagggggaacgaagtcagtcacgaggccgactaggtcatctgctgaaatcacttgtgaccttactgtaataaatgccttctacatccactggtacctacaccaggaggggaaggccccacagcgtcttctgtactatgacgtctccaactcaaaggatgtgttggaatcaggactcagtccaggaaagtattatactcatacacccaggaggtggagctggatattgatactacgaaatctaattgaaaatgattctggggtctattactgtgccacctgggacaggcctgagatttattataagaaactctttggcagtggaacaacactggttgtcacagataaacaacttgatgcagatgtttcccccaagcccactatttttcttccttcaattgctgaaacaaagctccagaaggctggaacatacctttgtcttcttgagaaatttttccctgatgttattaagatacattggcaagaaaagaagagcaacacgattctgggatcccaggaggggaacaccatgaagactaacgacacatacatgaaatttagctggttaacggtgccagaaaagtcactggacaaagaacacagatgtatcgtcagacatgagaataataaaaacggagttgatcaagaaattatctttcctccaataaagacagatgtcatcacaatggatcccaaagacaattgttcaaaagatgcaaatgatacactactgctgcagctcacaaacacctctgcatattacatgtacctcctcctgctcctcaagagtgtggtctattttgccatcatcacctgctgtctgcttagaagaacggctttctgctgcaatggagagaaatca

SEQ ID NO: 52 - DNA, 891 bp, Artificial
  TRD E113 codon opt.
atggccatgctgctgggagccagcgtgctgatcctgtggctgcagcccgattgggtcaacagccagcagaagaacgacgaccagcaagtgaagcagaacagccccagcctgagcgtgcaggaaggccggatcagcatcctgaactgcgactacaccaactctatgttcgactacttcctgtggtacaagaagtaccccgccgagggccccaccttcctgatctccatcagcagcatcaaggacaagaacgaggacggccggttcaccgtgtttctgaacaagagcgccaagcacctgagcctgcacatcgtgcctagccagcctggcgatagcgccgtgtacttttgtgccgccagcagccccatcagaggctacaccggcagcgacaagctgatcttcggcaagggcaccagagtgaccgtggaacccagaagccagccccacaccaagcccagcgtgttcgtgatgaagaacggcaccaacgtggcctgcctcgtgaaagagttctaccccaaggacatccggatcaacctggtgtccagcaagaagatcaccgagttcgaccccgccatcgtgatcagcccctccggcaagtacaacgccgtgaagctggggaagtacgaggacagcaacagcgtgacctgctccgtgcagcacgacaacaagaccgtgcacagcaccgatttcgaagtgaaaaccgactccaccgaccacgtgaagcccaaagagacagagaacaccaagcagcccagcaagagctgccacaagcccaaggccatcgtgcacaccgagaaagtgaacatgatgagcctgaccgtgctgggcctgcggatgctgttcgccaaaaccgtggccgtgaacttcctgctgaccgccaagctgttctttctg

SEQ ID NO: 53 - DNA, 924 bp, Artificial
  TRG E113 codon opt.
atggagtgggccctggccgtgctgctggcctttctgagccctgccagccagaagtccagcaacctggaaggccggaccaagagcgtgatccggcagacaggcagcagcgccgagatcacctgtgacctggccgagggcagcaccggctacatccactggtatctgcaccaagaaggcaaggccccccagcggctgctgtactacgacagctacaccagctccgtggtgctggaaagcggcatcagccccgggaagtacgacacctacggcagcacccggaagaacctgcggatgatcctgcggaacctgatcgagaacgacagcggcgtgtactactgcgccacctgggacggccccccctactacaagaagctgttcggcagcggcaccaccctggtggtgacagacaagcagctggacgccgacgtgtcccccaagcctaccatcttcctgccctcaattgctgagacaaagctgcagaaggccggcacctacctgtgcctgctggaaaagttcttcccagacgtgatcaagatccactgggaggaaaagaagtccaacaccatcctgggcagccaagaaggcaacaccatgaagaccaacgacacctacatgaagttcagctggctgaccgtgcccgagaagtccctggacaaagaacaccggtgcatcgtgcggcacgagaacaacaagaacggcgtggaccaagaaatcatcttcccacccatcaagaccgacgtgatcacaatggaccccaaggacaactgcagcaaggacgccaacgataccctgctgctgcagctgacaaacaccagcgcctactacatgtacttgttgctgctgctgaagtccgtggtgtacttcgccatcatcacatgctgcctgctgcggcggaccgccttctgctgcaacggcgagaagtcc

SEQ ID NO: 54 - DNA, 873 bp, Artificial
  TRD F4 codon opt.
atggtgttcagcagcctgctgtgcgtgttcgtggccttcagctacagcggcagcagcgtggcccagaaagtgacccaggcccagagcagcgtgtccatgcctgtgcggaaggccgtgaccctgaactgcctgtacgagacaagctggtggtcctactacatcttctggtacaagcagctgcccagcaaagagatgatcttcctgatccggcagggcagcgacgagcagaacgccaagagcggccggtacagcgtgaacttcaagaaagccgccaagtccgtggccctgaccatcagcgccctgcagctggaagatagcgccaagtacttctgcgccctgggcgagctgcgatattggggaatcgtggacaagctgatcttcggcaagggcaccagagtgaccgtggaacccagaagccagccccacaccaagccctccgtgttcgtgatgaagaacggcaccaacgtggcctgcctggtgaaagaattctaccccaaggacatccggatcaacctggtgtccagcaagaagatcaccgagttcgaccccgccatcgtgatcagccccagcggcaagtacaacgccgtgaagctggggaagtacgaggacagcaacagcgtgacctgcagcgtgcagcacgacaacaagaccgtgcacagcaccgacttcgaagtgaaaaccgactccaccgaccacgtgaagcccaaagagacagagaacaccaagcagcccagcaagagctgccacaagcccaaggccatcgtgcacaccgagaaagtgaacatgatgagcctgaccgtgctgggcctgcggatgctgttcgccaagacagtggccgtgaacttcctgctgaccgccaagctgttctttctg

SEQ ID NO: 55 - DNA, 915 bp, Artificial
  TRG F4 codon opt.
atggagtgggcactcgcagtgttgctcgcttttttgtctcctgcctcccagaagtctagtaacctggaggggcggactaagtccgtcattaggcagactggtagcagtgccgagattacctgcgacttggctgaaggcagcaatggctacatccactggtacttgcaccaagaaggcaaagcaccgcagcgactgcaatattatgactcctacaactcaaaggttgtgctcgaaagtggagtctctcccggcaagtattacacttacgcaagcacccgaaataatttgcgacttatcctgagaaacctgatagaaaatgatagcggcgtgtactactgcgccacctgggacggccaaaagaagctgttcggcagcggcaccaccctggtggtgacagacaagcagctggacgccgacgtgtcccccaagcctaccatcttcctgccctcaattgctgagacaaagctgcagaaggccggcacctacctgtgcctgctggaaaagttcttcccagacgtgatcaagatccactgggaggaaaagaagtccaacaccatcctgggcagccaagaaggcaacaccatgaagaccaacgacacctacatgaagttcagctggctgaccgtgcccgagaagtccctggacaaagaacaccggtgcatcgtgcggcacgagaacaacaagaacggcgtggaccaagaaatcatcttcccacccatcaagaccgacgtgatcacaatggaccccaaggacaactgcagcaaggacgccaacgataccctgctgctgcagctgacaaacaccagcgcctactacatgtacttgttgctgctgctgaagtccgtggtgtacttcgccatcatcacatgctgcctgctgcggcggaccgccttctgctgcaacggcgagaagtcc

SEQ ID NO: 56 - DNA, 897 bp, Artificial
  TRDZi11 codon opt.
atggtctttagcagcctgctgtgcgtgttcgtggccttcagctacagcggcagcagcgtggcccagaaagtgacacaggctcagagcagcgtgtccatgcctgtgcggaaggccgtgaccctgaactgcctgtacgagacaagctggtggtcctactacatcttctggtacaagcagctgcccagcaaagagatgatcttcctgatccggcagggcagcgacgagcagaatgccaagagcggccggtacagcgtgaacttcaagaaagccgccaagtccgtggccctgaccatctctgctctgcagctggaagatagcgccaagtacttctgcgccctgggcgagctgagaggccagatcagcttcctgtacctgctgggcgacaccaccgacaagctgattttcggcaagggcaccagagtgaccgtggaacccagaagccagccccacaccaagccctccgtgtttgtgatgaagaacggcaccaacgtggcctgcctcgtgaaagagttctaccccaaggacatccggatcaacctggtgtccagcaagaagatcaccgagttcgaccccgccatcgtgatcagccccagcggcaagtacaacgccgtgaagctggggaagtacgaggacagcaacagcgtgacctgcagcgtgcagcacgacaacaagaccgtgcacagcaccgatttcgaagtgaaaaccgactccaccgaccacgtgaagcccaaagagacagagaacaccaagcagcccagcaagagctgccacaagcccaaggccatcgtgcacaccgagaaagtgaacatgatgagcctgaccgtgctgggcctgcggatgctgttcgccaaaaccgtggccgtgaatttcctgctgaccgccaagctgttctttctg

SEQ ID NO: 57 - DNA, 915 bp, Artificial
  TRG Zi11 codon opt
atggtgctggctctggctctgctgctggcctttctgcctcccgccagccagaagtccagcaacctggaaggccggaccaagagcgtgaccagacctacaggatctagcgccgtgatcacctgtgacctgcccgtggaaaacgccgtgtacacccactggtatctgcaccaggaaggcaaggccccccagcggctgctgtactacgacagctacaacagccgggtggtgctggaaagcggcatcagcagagagaagtaccacacctacgccagcaccggcaagagcctgaagttcatcctggaaaacctgatcgagcgggactccggcgtgtactactgcgccacctgggacaactacaagaagctgttcggcagcggcaccaccctggtcgtgaccgacaaacagctggacgccgacgtgtcccccaagcctaccatcttcctgccctctatcgccgagacaaagctgcagaaggccggcacctacctgtgcctgctggaaaagttcttcccagacgtgatcaagatccactggcaggaaaagaagtccaacaccatcctgggcagccaggaagggaacaccatgaagaccaacgacacctacatgaagttcagctggctgaccgtgcccgagaagtccctggacaaagaacaccggtgcatcgtgcggcacgagaacaacaagaacggcgtggaccaggaaatcatcttcccacccatcaagaccgatgtgatcactatggaccccaaggacaactgcagcaaggacgccaacgataccctgctgctgcagctgaccaacaccagcgcctactacatgtatttgttgctgctgctgaagtccgtggtgtacttcgccatcatcacatgctgcctgctgcggcggaccgccttctgctgcaatggcgagaagtct

SEQ ID NO: 58 - DNA, 891 bp, Artificial; identical to SEQ ID NO: 52
  TRD D37 codon opt

SEQ ID NO: 59 - DNA, 915 bp, Artificial
  TRG D37 codon opt.
atggtgctggccctggctctgctgctggcctttctgccccctgccagccagaagtccagcaacctggaaggccggaccaagagcgtgaccagacctaccggcagcagcgccgtgatcacctgtgacctgcccgtggaaaacgccgtgtacacccactggtatctgcaccaagaaggcaaggccccccagcggctgctgtactacgacagctacaacagccgggtggtgctggaaagcggcatcagcagagagaagtaccacacctacgccagcaccggcaagagcctgaagttcatcctggaaaacctgatcgagcgggacagcggcgtgtactactgcgccacctgggacaattacatgaagttgtttgggtctgggactacattggttgtaactgacaagcagctggacgccgacgtgtcccccaagcctaccatcttcctgccctcaattgctgagacaaagctgcagaaggccggcacctacctgtgcctgctggaaaagttcttcccagacgtgatcaagatccactgggaggaaaagaagtccaacaccatcctgggcagccaagaaggcaacaccatgaagaccaacgacacctacatgaagttcagctggctgaccgtgcccgagaagtccctggacaaagaacaccggtgcatcgtgcggcacgagaacaacaagaacggcgtggaccaagaaatcatcttcccacccatcaagaccgacgtgatcacaatggaccccaaggacaactgcagcaaggacgccaacgataccctgctgctgcagctgacaaacaccagcgcctactacatgtacttgttgctgctgctgaagtccgtggtgtacttcgccatcatcacatgctgcctgctgcggcggaccgccttctgctgcaacggcgagaagtcc

SEQ ID NO: 60 - DNA, 891 bp, Artificial; identical to SEQ ID NO: 52
  TRD C132 codon opt.

SEQ ID NO: 61 - DNA, 921 bp, Artificial
  TRG C132 codon opt.
atggagtgggccctggccgtgctgctggcctttctgagccctgccagccagaagtccagcaacctggaaggccggaccaagagcgtgatccggcagacaggcagcagcgccgagatcacctgtgacctggccgagggcagcaccggctacatccactggtatctgcaccaagaaggcaaggccccccagcggctgctgtactacgacagctacaccagctccgtggtgctggaaagcggcatcagccccgggaagtacgacacctacggcagcacccggaagaacctgcggatgatcctgcggaacctgatcgagaacgacagcggcgtgtactactgcgccacctgggacggcttctactacaagaagctgttcggcagcggcaccaccctggtggtgacagacaagcagctggacgccgacgtgtcccccaagcctaccatcttcctgccctcaattgctgagacaaagctgcagaaggccggcacctacctgtgcctgctggaaaagttcttcccagacgtgatcaagatccactgggaggaaaagaagtccaacaccatcctgggcagccaagaaggcaacaccatgaagaccaacgacacctacatgaagttcagctggctgaccgtgcccgagaagtccctggacaaagaacaccggtgcatcgtgcggcacgagaacaacaagaacggcgtggaccaagaaatcatcttcccacccatcaagaccgacgtgatcacaatggaccccaaggacaactgcagcaaggacgccaacgataccctgctgctgcagctgacaaacaccagcgcctactacatgtacttgttgctgctgctgaagtccgtggtgtacttcgccatcatcacatgctgcctgctgcggcggaccgccttctgctgcaacggcgagaagtcc

SEQ ID NO: 62 - DNA, 882 bp, Artificial
  TRD Fe11 codon opt.
atggtgttcagcagcctgctgtgcgtgttcgtggccttcagctacagcggcagcagcgtggcccagaaagtgacccaggcccagagcagcgtgtccatgcctgtgcggaaggccgtgaccctgaactgcctgtacgagacaagctggtggtcctactacatcttctggtacaagcagctgcccagcaaagagatgatcttcctgatccggcagggcagcgacgagcagaacgccaagagcggccggtacagcgtgaacttcaagaaagccgccaagtccgtggccctgaccatcagcgccctgcagctggaagatagcgccaagtacttctgcgccctgggcgacagctacggcggaggccccctgtacaccgacaagctgatcttcggcaagggcaccagagtgaccgtggaacccagaagccagccccacaccaagccctccgtgttcgtgatgaagaacggcaccaacgtggcctgcctggtcaaagaattctaccccaaggacatccggatcaacctggtgtccagcaagaagatcaccgagttcgaccccgccatcgtgatcagccccagcggcaagtacaacgccgtgaagctggggaagtacgaggacagcaacagcgtgacctgcagcgtgcagcacgacaacaagaccgtgcacagcaccgacttcgaagtgaaaaccgactccaccgaccacgtgaagcccaaagagacagagaacaccaagcagcccagcaagagctgccacaagcccaaggccatcgtgcacaccgagaaagtgaacatgatgagcctgaccgtgctgggcctgcggatgctgttcgccaagacagtggccgtgaacttcctgctgaccgccaagctgttctttctgtga

SEQ ID NO: 63 - DNA, 930 bp, Artificial
  TRG Fe11 codon opt.
atgggatgggccctgctggtgctgctggccttcctgagccctgccagccagaagtccagcaacctggaaggcggcaccaagagcgtgacccggcctaccagaagcagcgccgagatcacctgtgacctgaccgtgatcaacgccttctacatccactggtatctgcaccaggaaggcaaggccccccagcggctgctgtactacgacgtgtccaacagcaaggacgtgctggaaagcggcctgagccccggcaagtactacacccacacccccagacggtggtcctggattctgatcctgcggaacctgatcgagaacgacagcggcgtgtactactgcgccacctgggaccggcccgagatctactacaagaagctgttcggcagcggcaccaccctggtcgtgacagacaagcagctggacgccgacgtgtcccccaagcctaccatcttcctgccctcaattgctgagacaaagctgcagaaggccggcacctacctgtgcctgctggaaaagttcttcccagacgtgatcaagatccactgggaggaaaagaagtccaacaccatcctgggcagccaagaaggcaacaccatgaagaccaacgacacctacatgaagttcagctggctgaccgtgcccgagaagtccctggacaaagaacaccggtgcatcgtgcggcacgagaacaacaagaacggcgtggaccaagaaatcatcttcccacccatcaagaccgacgtgatcacaatggaccccaaggacaactgcagcaaggacgccaacgataccctgctgctgcagctgacaaacaccagcgcctactacatgtacttgttgctgctgctgaagtccgtggtgtacttcgccatcatcacatgctgcctgctgcggcggaccgccttctgctgcaacggcgagaagtcctga

SEQ ID NO: 64 - protein, 15 aa, Artificial
  Longer CDR3 VG5 Fe11
CATWDRPEIYYKKLF

SEQ ID NO: 65 - protein, 14 aa, Artificial
  CDR3 VG4 F2
CATWDGPPYYKKLF

SEQ ID NO: 66 - protein, 26 aa, Artificial
  CDR3 VD1 Ze11
CALGDYLGDKYPSYDLLGDTTDKLIF

SEQ ID NO: 67 - protein, 11 aa, Artificial
  CDR3 VG8 Ze11
CATWDNYKKLF

SEQ ID NO: 68 - protein, 18 aa, Artificial
  CDR3 VD5 B23
CAASSPIRGYTGSDKLIF

SEQ ID NO: 69 - protein, 11 aa, Artificial
  CDR3 VG8 B23
CATWDNYKKLF

SEQ ID NO: 70 - protein, 280 aa, Homo sapiens
CDKVTQSSPDQTVASGSEVVLLCTYDTVYSNPDLFWYRIRPDYSFQFVFYGDNSRSEGADFTQGRFSVKHILTQKAFHLVISPVRTEDSATYYCASSYTLKLGDTPGRVRDWKLIFGKGTRVTVEPRSQPHTKPSVFVMKNGTNVACLVKEFYPKDIRINLVSSKKITEFDPAIVISPSGKYNAVKLGKYEDSNSVTCSVQHDNKTVHSTDFEVKTDSTDHVKPKETENTKQPSKSCHKPKAIVHTEKVNMMSLTVLGLRMLFAKTVAVNFLLTAKLFFL

SEQ ID NO: 71 - protein, 290 aa, Homo sapiens; identical to SEQ ID NO: 30

SEQ ID NO: 72 - protein, 280 aa, Homo sapiens
AQKVTQAQSSVSMPVRKAVTLNCLYETSWWSYYIFWYKQLPSKEMIFLIRQGSDEQNAKSGRYSVNFKKAAKSVALTISALQLEDSAKYFCALGDYLGDKYPSYDLLGDTTDKLIFGKGTRVTVEPRSQPHTKPSVFVMKNGTNVACLVKEFYPKDIRINLVSSKKITEFDPAIVISPSGKYNAVKLGKYEDSNSVTCSVQHDNKTVHSTDFEVKTDSTDHVKPKETENTKQPSKSCHKPKAIVHTEKVNMMSLTVLGLRMLFAKTVAVNFLLTAKLFFL

SEQ ID NO: 73 - protein, 287 aa, Homo sapiens; identical to SEQ ID NO: 34

SEQ ID NO: 74 - protein, 271 aa, Homo sapiens; identical to SEQ ID NO: 29

SEQ ID NO: 75 - protein, 287 aa, Homo sapiens; identical to SEQ ID NO: 34

SEQ ID NO: 76 - DNA, 895 bp, Homo sapiens
atgattcttactgtgggctttagctttttgtttttctacaggggcacgctgtgtgacaaagtaacccagagttccccggaccagacggtggcgagtggcagtgaggtggtactgctctgcacttacgacactgtatattcaaatccagatttattctggtaccggataaggccagattattcctttcagtttgtcttttatggggataacagcagatcagaaggtgcagattttactcaaggacggttttctgtgaaacacattctgacccagaaagcctttcacttggtgatctctccagtaaggactgaagacagtgccacttactactgtgcctcctcctatactctcaaactgggggatacgccgggtagggtccgtgattggaaactcatctttggaaaaggaacccgtgtgactgtggaaccaagaagtcagcctcataccaaaccatccgtttttgtcatgaaaaatggaacaaatgtcgcttgtctggtgaaggaattctaccccaaggatataagaataaatctcgtgtcatccaagaagataacagagtttgatcctgctattgtcatctctcccagtgggaagtacaatgctgtcaagcttggtaaatatgaagattcaaattcagtgacatgttcagttcaacacgacaataaaactgtgcactccactgactttgaagtgaagacagattctacagatcacgtaaaaccaaaggaaactgaaaacacaaagcaaccttcaaagagctgccataaacccaaagccatagttcataccgagaaggtgaacatgatgtccctcacagtgcttgggctacgaatgctgtttgcaaagactgttgccgtcaattttctcttgactgccaagttatttttcttgtaag

SEQ ID NO: 77 - DNA, 924 bp, Homo sapiens; identical to SEQ ID NO: 41

SEQ ID NO: 78 - DNA, 904 bp, Homo sapiens
atgctgttctccagcctgctgtgtgtatttgtggccttcagctactctggatcaagtgtggcccagaaggttactcaagcccagtcatcagtatccatgccagtgaggaaagcagtcaccctgaactgcctgtatgaaacaagttggtggtcatattatattttttggtacaagcaacttcccagcaaagagatgattttccttattcgccagggttctgatgaacagaatgcaaaaagtggtcgctattctgtcaacttcaagaaagcagcgaaatccgtcgccttaaccatttcagccttacagctagaagattcagcaaagtacttttgtgctcttggggactatttaggggacaaatatccttcctacgatttactgggggatacaaccgataaactcatctttggaaaaggaacccgtgtgactgtggaaccaagaagtcagcctcataccaaaccatccgtttttgtcatgaaaaatggaacaaatgtcgcttgtctggtgaaggaattctaccccaaggatataagaataaatctcgtgtcatccaagaagataacagagtttgatcctgctattgtcatctctcccagtgggaagtacaatgctgtcaagcttggtaaatatgaagattcaaattcagtgacatgttcagttcaacacgacaataaaactgtgcactccactgactttgaagtgaagacagattctacagatcacgtaaaaccaaaggaaactgaaaacacaaagcaaccttcaaagagctgccataaacccaaagccatagttcataccgagaaggtgaacatgatgtccctcacagtgcttgggctacgaatgctgtttgcaaagactgttgccgtcaattttctcttgactgccaagttatttttcttgtaag

SEQ ID NO: 79 - DNA, 915 bp, Homo sapiens; identical to SEQ ID NO: 45

SEQ ID NO: 80 - DNA, 895 bp, Homo sapiens; identical to SEQ ID NO: 26

SEQ ID NO: 81 - DNA, 915 bp, Homo sapiens; identical to SEQ ID NO: 45

SEQ ID NO: 82 - DNA, 891 bp, Artificial
  TRD F2 codon opt.
atggttcttacagtaggattttctttcctcttcttctacagagggactctttgcgacaaagtgacacaaagcagtccggaccaaacggtggcgtctggttccgaagtggtgcttctttgcacttatgatacggtatatagcaatccggacctcttctggtatcgcatacgcccggattatagttttcaattcgtcttctatggcgacaactctcgaagcgaaggcgcagattttacccaggggcgcttttcagttaaacacatattgacccagaaggcttttcacttggtgatctctcctgtgagaactgaggattccgcgacttattactgcgcgtcttcttacacccttaaattgggggacacgccaggcagagtccgcgactggaagctgatcttcggcaagggcaccagagtgaccgtggaacccagaagccagccccacaccaagccctccgtgttcgtgatgaagaacggcaccaacgtggcctgcctggtgaaagaattctaccccaaggacatccggatcaacctggtgtccagcaagaagatcaccgagttcgaccccgccatcgtgatcagccccagcggcaagtacaacgccgtgaagctggggaagtacgaggacagcaacagcgtgacctgcagcgtgcagcacgacaacaagaccgtgcacagcaccgacttcgaagtgaaaaccgactccaccgaccacgtgaagcccaaagagacagagaacaccaagcagcccagcaagagctgccacaagcccaaggccatcgtgcacaccgagaaagtgaacatgatgagcctgaccgtgctgggcctgcggatgctgttcgccaagacagtggccgtgaacttcctgctgaccgccaagctgttctttctg

SEQ ID NO: 83 - DNA, 924 bp, Artificial; identical to SEQ ID NO: 53
  TRG F2 codon opt.

SEQ ID NO: 84 - DNA, 900 bp, Artificial
  TRD Ze 11 codon opt.
atggtgttcagcagcctgctgtgcgtgttcgtggccttcagctacagcggcagcagcgtggcccagaaagtgacacaggctcagagcagcgtgtccatgcctgtgcggaaggccgtgaccctgaactgcctgtacgagacaagctggtggtcctactacatcttctggtacaagcagctgcccagcaaagagatgatcttcctgatccggcagggcagcgacgagcagaatgccaagagcggccggtacagcgtgaacttcaagaaagccgccaagtccgtggccctgaccatctctgctctgcagctggaagatagcgccaagtacttctgcgccctgggcgactacctgggcgataagtaccccagctacgacctgctgggcgacaccaccgacaagctgatcttcggcaagggcaccagagtgaccgtggaacccagaagccagccccacaccaagccctccgtgtttgtgatgaagaacggcaccaacgtggcctgcctcgtgaaagagttctaccccaaggacatccggatcaacctggtgtccagcaagaagatcaccgagttcgaccccgccatcgtgatcagccccagcggcaagtacaacgccgtgaagctggggaagtacgaggacagcaacagcgtgacctgcagcgtgcagcacgacaacaagaccgtgcacagcaccgatttcgaagtgaaaaccgactccaccgaccacgtgaagcccaaagagacagagaacaccaagcagcccagcaagagctgccacaagcccaaggccatcgtgcacaccgagaaagtgaacatgatgagcctgaccgtgctgggcctgcggatgctgttcgccaaaaccgtggccgtgaatttcctgctgaccgccaagctgttctttctg

SEQ ID NO: 85 - DNA, 915 bp, Artificial; identical to SEQ ID NO: 57
  TRG Ze11 codon opt.

SEQ ID NO: 86 - DNA, 891 bp, Artificial; identical to SEQ ID NO: 52
  TRD B23 codon opt.

SEQ ID NO: 87 - DNA, 915 bp, Artificial; identical to SEQ ID NO: 57
  TRG B23 codon opt.

SEQ ID NO: 88 - protein, 20 aa, Artificial
  CDR3 VD1 B9
CALGNGNHIGYWRYTDKLIF

SEQ ID NO: 89 - protein, 13 aa, Artificial
  CDR3 VG5  B9
CATWDRLYYKKLF

SEQ ID NO: 90 - protein, 274 aa, Homo sapiens
AQKVTQAQSSVSMPVRKAVTLNCLYETSWWSYYIFWYKQLPSKEMIFLIRQGSDEQNAKSGRYSVNFKKAAKSVALTISALQLEDSAKYFCALGNGNHIGYWRYTDKLIFGKGTRVTVEPRSQPHTKPSVFVMKNGTNVACLVKEFYPKDIRINLVSSKKITEFDPAIVISPSGKYNAVKLGKYEDSNSVTCSVQHDNKTVHSTDFEVKTDSTDHVKPKETENTKQPSKSCHKPKAIVHTEKVNMMSLTVLGLRMLFAKTVAVNFLLTAKLFFL

SEQ ID NO: 91 - protein, 289 aa, Homo sapiens
SSNLEGGTKSVTRPTRSSAEITCDLTVINAFYIHWYLHQEGKAPQRLLYYDVSNSKDVLESGLSPGKYYTHTPRRWSWILILRNLIENDSGVYYCATWDRLYYKKLFGSGTTLVVTDKQLDADVSPKPTIFLPSIAETKLQKAGTYLCLLEKFFPDVIKIHWEEKKSNTILGSQEGNTMKTNDTYMKFSWLTVPEKSLDKEHRCIVRHENNKNGVDQEIIFPPIKTDVITMDPKDNCSKDANDTLLLQLTNTSAYYMYLLLLLKSVVYFAIITCCLLRRTAFCCNGEKS

SEQ ID NO: 92 - DNA, 886 bp, Homo sapiens
atgctgttctccagcctgctgtgtgtatttgtggccttcagctactctggatcaagtgtggcccagaaggttactcaagcccagtcatcagtatccatgccagtgaggaaagcagtcaccctgaactgcctgtatgaaacaagttggtggtcatattatattttttggtacaagcaacttcccagcaaagagatgattttccttattcgccagggttctgatgaacagaatgcaaaaagtggtcgctattctgtcaacttcaagaaagcagcgaaatccgtcgccttaaccatttcagccttacagctagaagattcagcaaagtacttttgtgctcttggaaacggtaatcacatcgggtactggcggtacaccgataaactcatctttggaaaaggaacccgtgtgactgtggaaccaagaagtcagcctcataccaaaccatccgtttttgtcatgaaaaatggaacaaatgtcgcttgtctggtgaaggaattctaccccaaggatataagaataaatctcgtgtcatccaagaagataacagagtttgatcctgctattgtcatctctcccagtgggaagtacaatgctgtcaagcttggtaaatatgaagattcaaattcagtgacatgttcagttcaacacgacaataaaactgtgcactccactgactttgaagtgaagacagattctacagatcacgtaaaaccaaaggaaactgaaaacacaaagcaaccttcaaagagctgccataaacccaaagccatagttcataccgagaaggtgaacatgatgtccctcacagtgcttgggctacgaatgctgtttgcaaagactgttgccgtcaattttctcttgactgccaagttatttttcttgtaag

SEQ ID NO: 93 - DNA, 921 bp, Homo sapiens
atgcggtgggccctactggtgcttctagctttcctgtctcctgccagtcagaaatcttccaacttggaagggggaacgaagtcagtcacgaggccgactaggtcatctgctgaaatcacttgtgaccttactgtaataaatgccttctacatccactggtacctacaccaggaggggaaggccccacagcgtcttctgtactatgacgtctccaactcaaaggatgtgttggaatcaggactcagtccaggaaagtattatactcatacacccaggaggtggagctggatattgatactacgaaatctaattgaaaatgattctggggtctattactgtgccacctgggacagactttattataagaaactctttggcagtggaacaacactggttgtcacagataaacaacttgatgcagatgtttcccccaagcccactatttttcttccttcaattgctgaaacaaagctccagaaggctggaacatacctttgtcttcttgagaaatttttccctgatgttattaagatacattggcaagaaaagaagagcaacacgattctgggatcccaggaggggaacaccatgaagactaacgacacatacatgaaatttagctggttaacggtgccagaaaagtcactggacaaagaacacagatgtatcgtcagacatgagaataataaaaacggagttgatcaagaaattatctttcctccaataaagacagatgtcatcacaatggatcccaaagacaattgttcaaaagatgcaaatgatacactactgctgcagctcacaaacacctctgcatattacatgtacctcctcctgctcctcaagagtgtggtctattttgccatcatcacctgctgtctgcttagaagaacggctttctgctgcaatggagagaaatca

SEQ ID NO: 94 - DNA, 882 bp, Artificial
  TRD B9 codon opt.
atggtgttcagcagcctgctgtgcgtgttcgtggccttcagctacagcggcagcagcgtggcccagaaagtgacccaggcccagagcagcgtgtccatgcctgtgcggaaggccgtgaccctgaactgcctgtacgagacaagctggtggtcctactacatcttctggtacaagcagctgcccagcaaagagatgatcttcctgatccggcagggcagcgacgagcagaacgccaagagcggccggtacagcgtgaacttcaagaaagccgccaagtccgtggccctgaccatcagcgccctgcagctggaagatagcgccaagtacttctgcgccctgggcaatggcaatcatattggatactggcgatataccgacaagctgatcttcggcaagggcaccagagtgaccgtggaacccagaagccagccccacaccaagccctccgtgttcgtgatgaagaacggcaccaacgtggcctgcctggtgaaagaattctaccccaaggacatccggatcaacctggtgtccagcaagaagatcaccgagttcgaccccgccatcgtgatcagccccagcggcaagtacaacgccgtgaagctggggaagtacgaggacagcaacagcgtgacctgcagcgtgcagcacgacaacaagaccgtgcacagcaccgacttcgaagtgaaaaccgactccaccgaccacgtgaagcccaaagagacagagaacaccaagcagcccagcaagagctgccacaagcccaaggccatcgtgcacaccgagaaagtgaacatgatgagcctgaccgtgctgggcctgcggatgctgttcgccaagacagtggccgtgaacttcctgctgaccgccaagctgttctttctg

SEQ ID NO: 95 - DNA, 921 bp, Artificial
  TRG B9 codon opt.
atggtgtgggccctgctggtgctgctggccttcctgagccccgccagccagaagagcagcaacctggagggcggcaccaagagcgtgacccggcccacccggagcagcgccgagatcacctgcgacctgaccgtgatcaacgccttctacatccactggtatctgcaccaggagggcaaggccccccagcggctgctgtactacgacgtgagcaacagcaaggacgtgctggagagcggcctgagccccggcaagtactacacccacaccccccggcggtggagctggattctgatcctgcggaacctgatcgagaacgacagcggcgtgtactactgcgccacctgggaccggctgtactacaagaagctgttcggcagcggcaccaccctggtggtgaccgacaagcagctggacgccgacgtgtcccccaagcctaccatcttcctgccctcaattgctgagacaaagctgcagaaggccggcacctacctgtgcctgctggaaaagttcttcccagacgtgatcaagatccactgggaggaaaagaagtccaacaccatcctgggcagccaagaaggcaacaccatgaagaccaacgacacctacatgaagttcagctggctgaccgtgcccgagaagtccctggacaaagaacaccggtgcatcgtgcggcacgagaacaacaagaacggcgtggaccaagaaatcatcttcccacccatcaagaccgacgtgatcacaatggaccccaaggacaactgcagcaaggacgccaacgataccctgctgctgcagctgacaaacaccagcgcctactacatgtacttgttgctgctgctgaagtccgtggtgtacttcgccatcatcacatgctgcctgctgcggcggaccgccttctgctgcaacggcgagaagtcc

SEQ ID NO: 96 - protein, 273 aa, Homo sapiens
AQKVTQAQSSVSMPVRKAVTLNCLYETSWWSYYIFWYKQLPSKEMIFLIRQGSDEQNAKSGRYSVNFKKAAKSVALTISALQLEDSAKYFCALGDSYGGGPLYTDKLIFGKGTRVTVEPRSQPHTKPSVFVMKNGTNVACLVKEFYPKDIRINLVSSKKITEFDPAIVISPSGKYNAVKLGKYEDSNSVTCSVQHDNKTVHSTDFEVKTDSTDHVKPKETENTKQPSKSCHKPKAIVHTEKVNMMSLTVLGLRMLFAKTVAVNFLLTAKLFFL

SEQ ID NO: 97 - protein, 291 aa, Homo sapiens
SSNLEGGTKSVTRPTRSSAEITCDLTVINAFYIHWYLHQEGKAPQRLLYYDVSNSKDVLESGLSPGKYYTHTPRRWSWILILRNLIENDSGVYYCATWDRPEIYYKKLFGSGTTLVVTDKQLDADVSPKPTIFLPSIAETKLQKAGTYLCLLEKFFPDVIKIHWEEKKSNTILGSQEGNTMKTNDTYMKFSWLTVPEKSLDKEHRCIVRHENNKNGVDQEIIFPPIKTDVITMDPKDNCSKDANDTLLLQLTNTSAYYMYLLLLLKSVVYFAIITCCLLRRTAFCCNGEKS

SEQ ID NO: 98 - protein, 269 aa, Homo sapiens
AIELVPEHQTVPVSIGVPATLRCSMKGEAIGNYYINWYRKTQGNTMTFIYREKDIYGPGFKDNFQGDIDIAKNLAVLKILAPSERDEGSYYCACDLLGYTDKLIFGKGTRVTVEPRSQPHTKPSVFVMKNGTNVACLVKEFYPKDIRINLVSSKKITEFDPAIVISPSGKYNAVKLGKYEDSNSVTCSVQHDNKTVHSTDFEVKTDSTDHVKPKETENTKQPSKSCHKPKAIVHTEKVNMMSLTVLGLRMLFAKTVAVNFLLTAKLFFL

SEQ ID NO: 99 - protein, 293 aa, Homo sapiens
AGHLEQPQISSTKTLSKTARLECVVSGITISATSVYWYRERPGEVIQFLVSISYDGTVRKESGIPSGKFEVDRIPETSTSTLTIHNVEKQDIATYYCALWEEELGKKIKVFGPGTKLIITDKQLDADVSPKPTIFLPSIAETKLQKAGTYLCLLEKFFPDVIKIHWEEKKSNTILGSQEGNTMKTNDTYMKFSWLTVPEKSLDKEHRCIVRHENNKNGVDQEIIFPPIKTDVITMDPKDNCSKDANDTLLLQLTNTSAYYMYLLLLLKSVVYFAIITCCLLRRTAFCCNGEKS

SEQ ID NO: 100 - protein, 271 aa, Homo sapiens
AIELVPEHQTVPVSIGVPATLRCSMKGEAIGNYYINWYRKTQGNTMTFIYREKDIYGPGFKDNFQGDIDIAKNLAVLKILAPSERDEGSYYCACDALKRTDTDKLIFGKGTRVTVEPRSQPHTKPSVFVMKNGTNVACLVKEFYPKDIRINLVSSKKITEFDPAIVISPSGKYNAVKLGKYEDSNSVTCSVQHDNKTVHSTDFEVKTDSTDHVKPKETENTKQPSKSCHKPKAIVHTEKVNMMSLTVLGLRMLFAKTVAVNFLLTAKLFFL

SEQ ID NO: 101 - protein, 294 aa, Homo sapiens
AGHLEQPQISSTKTLSKTARLECVVSGITISATSVYWYRERPGEVIQFLVSISYDGTVRKESGIPSGKFEVDRIPETSTSTLTIHNVEKQDIATYYCALWEIQELGKKIKVFGPGTKLIITDKQLDADVSPKPTIFLPSIAETKLQKAGTYLCLLEKFFPDVIKIHWEEKKSNTILGSQEGNTMKTNDTYMKFSWLTVPEKSLDKEHRCIVRHENNKNGVDQEIIFPPIKTDVITMDPKDNCSKDANDTLLLQLTNTSAYYMYLLLLLKSVVYFAIITCCLLRRTAFCCNGEKS